European Patent Specification EP 4 022 086 B1, published August 6, 2025. Title: COMPOSITIONS AND METHODS FOR AMPLIFICATION AND DETECTION OF HEPATITIS B VIRUS RNA, INCLUDING HBV RNA TRANSCRIBED FROM CCCDNA. Applicant: F. Hoffmann-La Roche AG Roche Diagnostics GmbH Roche Molecular Systems, Inc. The sequence listing filed with the application follows.

SEQUENCE LISTING (400 sequences)

SEQ ID NO: 1 - DNA, 23 bp, Artificial Sequence
  Description of Artificial Sequence: Synthetic primer
aactccacagaagctccaaattc

SEQ ID NO: 2 - DNA, 28 bp, Artificial Sequence
  Description of Artificial Sequence: Synthetic primer
agagtaactccacagaagctccaaattc

SEQ ID NO: 3 - DNA, 22 bp, Artificial Sequence
  Description of Artificial Sequence: Synthetic primer
gagagtaactccacagaagctc

SEQ ID NO: 4 - DNA, 20 bp, Artificial Sequence
  Description of Artificial Sequence: Synthetic primer
gagagtaactccacagaagc

SEQ ID NO: 5 - DNA, 20 bp, Artificial Sequence
  Description of Artificial Sequence: Synthetic primer
gagagtaactccacagaagc

SEQ ID NO: 6 - DNA, 34 bp, Artificial Sequence
  Description of Artificial Sequence: Synthetic primer
  modified_base (14)..(14): Inosine
cagaaggcaaaaangagagtaactccacagaagc

SEQ ID NO: 7 - DNA, 29 bp, Artificial Sequence
  Description of Artificial Sequence: Synthetic primer
  modified_base (9)..(9): Inosine
ggcaaaaangagagtaactccacagaagc

SEQ ID NO: 8 - DNA, 20 bp, Artificial Sequence
  Description of Artificial Sequence: Synthetic primer
  Description of Combined DNA/RNA Molecule: Synthetic primer
gagaguaacuccacagaagc

SEQ ID NO: 9 - DNA, 28 bp, Artificial Sequence
  Description of Artificial Sequence: Synthetic primer
  Description of Combined DNA/RNA Molecule: Synthetic primer
agagtaacuccacagaagctccaaautc

SEQ ID NO: 10 - DNA, 28 bp, Artificial Sequence
  Description of Artificial Sequence: Synthetic primer
  Description of Combined DNA/RNA Molecule: Synthetic primer
agaguaacuccacagaagcuccaaautc

SEQ ID NO: 11 - DNA, 29 bp, Artificial Sequence
  Description of Artificial Sequence: Synthetic primer
  Description of Combined DNA/RNA Molecule: Synthetic primer
gagaguaacuccacagaagctccaaautc

SEQ ID NO: 12 - DNA, 29 bp, Artificial Sequence
  Description of Artificial Sequence: Synthetic primer
  Description of Combined DNA/RNA Molecule: Synthetic primer
gagaguaacuccacagaagcuccaaautc

SEQ ID NO: 13 - DNA, 43 bp, Artificial Sequence
  Description of Artificial Sequence: Synthetic primer
  modified_base (14)..(14): Inosine
cagaaggcaaaaangagagtaactccacagaagctccaaattc

SEQ ID NO: 14 - DNA, 49 bp, Artificial Sequence
  Description of Artificial Sequence: Synthetic primer
  modified_base (14)..(14): Inosine
cagaaggcaaaaangagagtaactccacagaagctccaaattctttata

SEQ ID NO: 15 - DNA, 20 bp, Artificial Sequence
  Description of Artificial Sequence: Synthetic primer
gagagtaactccacagaagc

SEQ ID NO: 16 - DNA, 25 bp, Artificial Sequence
  Description of Artificial Sequence: Synthetic primer
ttttttttttttttttttgctggtg

SEQ ID NO: 17 - DNA, 28 bp, Artificial Sequence
  Description of Artificial Sequence: Synthetic probe
  Description of Combined DNA/RNA Molecule: Synthetic probe
  misc_feature (10)..(11): BHQ-2
tguacuaggaggctgtaggcataaattg

SEQ ID NO: 18 - DNA, 50 bp, Artificial Sequence
  Description of Artificial Sequence: Synthetic primer
gatcaacgtgtcaccgcctattctattttttttttttttttttgctggtg

SEQ ID NO: 19 - DNA, 50 bp, Artificial Sequence
  Description of Artificial Sequence: Synthetic primer
aactgctgcttaaatcttgctacccttttttttttttttttttgctggtg

SEQ ID NO: 20 - DNA, 22 bp, Artificial Sequence
  Description of Artificial Sequence: Synthetic primer
  Description of Combined DNA/RNA Molecule: Synthetic primer
utgaggcauactucaaagactg

SEQ ID NO: 21 - DNA, 35 bp, Artificial Sequence
  Description of Artificial Sequence: Synthetic blocker sequence
  modified_base (18)..(19): Inosine
gttgcatggtgctggtgnncagaccaatttatgcc

SEQ ID NO: 22 - DNA, 23 bp, Artificial Sequence
  Description of Artificial Sequence: Synthetic blocker sequence
  modified_base (11)..(12): Inosine
ggugcuggugnncagacccaauu

SEQ ID NO: 23 - DNA, 23 bp, Artificial Sequence
  Description of Artificial Sequence: Synthetic primer
actcttggactctcagcaatgtc

SEQ ID NO: 24 - DNA, 23 bp, Artificial Sequence
  Description of Artificial Sequence: Synthetic primer
actcttggactctctgtaatgtc

SEQ ID NO: 25 - DNA, 28 bp, Artificial Sequence
  Description of Artificial Sequence: Synthetic primer
ttttttttttttttttttgctggtgaac

SEQ ID NO: 26 - DNA, 28 bp, Artificial Sequence
  Description of Artificial Sequence: Synthetic primer
ttttttttttttttttttgctggtgcgc

SEQ ID NO: 27 - DNA, 53 bp, Artificial Sequence
  Description of Artificial Sequence: Synthetic primer
gatcaacgtgtcaccgcctattctattttttttttttttttttgctggtgaac

SEQ ID NO: 28 - DNA, 53 bp, Artificial Sequence
  Description of Artificial Sequence: Synthetic primer
gatcaacgtgtcaccgcctattctattttttttttttttttttgctggtgcgc

SEQ ID NO: 29 - DNA, 53 bp, Artificial Sequence
  Description of Artificial Sequence: Synthetic primer
aactgctgcttaaatcttgctacccttttttttttttttttttgctggtgaac

SEQ ID NO: 30 - DNA, 53 bp, Artificial Sequence
  Description of Artificial Sequence: Synthetic primer
aactgctgcttaaatcttgctacccttttttttttttttttttgctggtgcgc

SEQ ID NO: 31 - DNA, 41 bp, Artificial Sequence
  Description of Artificial Sequence: Synthetic probe
  misc_feature (7)..(8): BHQ-2
accgaccttgaggcatacttcaaagactgtgtgtttaaaga

SEQ ID NO: 32 - DNA, 41 bp, Artificial Sequence
  Description of Artificial Sequence: Synthetic probe
  misc_feature (7)..(8): BHQ-2
acctggatcgaagaatacatcaaagactgtgtatttaagga

SEQ ID NO: 33 - DNA, 51 bp, Artificial Sequence
  Description of Artificial Sequence: Synthetic primer
atagaagagctgtcgtagtctccgattttttttttttttttttgaagctcc

SEQ ID NO: 34 - DNA, 51 bp, Artificial Sequence
  Description of Artificial Sequence: Synthetic primer
gatcaacgtgtcaccgcctattctattttttttttttttttttgaagctcc

SEQ ID NO: 35 - DNA, 51 bp, Artificial Sequence
  Description of Artificial Sequence: Synthetic primer
aactgctgcttaaatcttgctacccttttttttttttttttttgaagctcc

SEQ ID NO: 36 - DNA, 25 bp, Artificial Sequence
  Description of Artificial Sequence: Synthetic primer
atagaagagctgtcgtagtctccga

SEQ ID NO: 37 - DNA, 25 bp, Artificial Sequence
  Description of Artificial Sequence: Synthetic primer
gatcaacgtgtcaccgcctattcta

SEQ ID NO: 38 - DNA, 25 bp, Artificial Sequence
  Description of Artificial Sequence: Synthetic primer
aactgctgcttaaatcttgctaccc

SEQ ID NO: 39 - DNA, 26 bp, Artificial Sequence
  Description of Artificial Sequence: Synthetic primer
ttttttttttttttttttgaagctcc

SEQ ID NO: 40 - DNA, 50 bp, Artificial Sequence
  Description of Artificial Sequence: Synthetic primer
gatcaacgtgtcaccgcctattctattttttttttttttttttgaagctc

SEQ ID NO: 41 - DNA, 50 bp, Artificial Sequence
  Description of Artificial Sequence: Synthetic primer
aactgctgcttaaatcttgctacccttttttttttttttttttgaagctc

SEQ ID NO: 42 - DNA, 25 bp, Artificial Sequence
  Description of Artificial Sequence: Synthetic primer
ttttttttttttttttttgaagctc

SEQ ID NO: 43 - DNA, 48 bp, Artificial Sequence
  Description of Artificial Sequence: Synthetic primer
gatcaacgtgtcaccgcctattctattttttttttttttttttgaagc

SEQ ID NO: 44 - DNA, 48 bp, Artificial Sequence
  Description of Artificial Sequence: Synthetic primer
aactgctgcttaaatcttgctacccttttttttttttttttttgaagc

SEQ ID NO: 45 - DNA, 23 bp, Artificial Sequence
  Description of Artificial Sequence: Synthetic primer
ttttttttttttttttttgaagc

SEQ ID NO: 46 - DNA, 48 bp, Artificial Sequence
  Description of Artificial Sequence: Synthetic primer
gatcaacgtgtcaccgcctattctatttttttttttttttgaagctcc

SEQ ID NO: 47 - DNA, 48 bp, Artificial Sequence
  Description of Artificial Sequence: Synthetic primer
aactgctgcttaaatcttgctaccctttttttttttttttgaagctcc

SEQ ID NO: 48 - DNA, 45 bp, Artificial Sequence
  Description of Artificial Sequence: Synthetic primer
gatcaacgtgtcaccgcctattctattttttttttttgaagctcc

SEQ ID NO: 49 - DNA, 45 bp, Artificial Sequence
  Description of Artificial Sequence: Synthetic primer
aactgctgcttaaatcttgctacccttttttttttttgaagctcc

SEQ ID NO: 50 - DNA, 51 bp, Artificial Sequence
  Description of Artificial Sequence: Synthetic primer
gatcaacgtgtcaccgcctattctattttttttttttttttttgtagctcc

SEQ ID NO: 51 - DNA, 48 bp, Artificial Sequence
  Description of Artificial Sequence: Synthetic primer
gatcaacgtgtcaccgcctattctattttttttttttttttttgtagc

SEQ ID NO: 52 - DNA, 26 bp, Artificial Sequence
  Description of Artificial Sequence: Synthetic primer
ttttttttttttttttttgtagctcc

SEQ ID NO: 53 - DNA, 23 bp, Artificial Sequence
  Description of Artificial Sequence: Synthetic primer
ttttttttttttttttttgtagc

SEQ ID NO: 54 - DNA, 26 bp, Artificial Sequence
  Description of Artificial Sequence: Synthetic primer
tttttttttttttttttttttttttg

SEQ ID NO: 55 - DNA, 26 bp, Artificial Sequence
  Description of Artificial Sequence: Synthetic primer
  Description of Combined DNA/RNA Molecule: Synthetic primer
tttttttttuuutttuuutttuuutg

SEQ ID NO: 56 - DNA, 26 bp, Artificial Sequence
  Description of Artificial Sequence: Synthetic primer
  Description of Combined DNA/RNA Molecule: Synthetic primer
ttuuutttuuutttuuutgaagctcc

SEQ ID NO: 57 - DNA, 26 bp, Artificial Sequence
  Description of Artificial Sequence: Synthetic primer
  Description of Combined DNA/RNA Molecule: Synthetic primer
uuuuuuuuuuuuuuuuuugaagctcc

SEQ ID NO: 58 - DNA, 26 bp, Artificial Sequence
  Description of Artificial Sequence: Synthetic primer
  Description of Combined DNA/RNA Molecule: Synthetic primer
ttutttutttutttttttgaagctcc

SEQ ID NO: 59 - DNA, 26 bp, Artificial Sequence
  Description of Artificial Sequence: Synthetic primer
  Description of Combined DNA/RNA Molecule: Synthetic primer
ttuuutttuuutttuuutgaagctcc

SEQ ID NO: 60 - DNA, 26 bp, Artificial Sequence
  Description of Artificial Sequence: Synthetic primer
ttttttttttttttttttgaagctcc

SEQ ID NO: 61 - DNA, 25 bp, Artificial Sequence
  Description of Artificial Sequence: Synthetic primer
ttttttttttttttttttgaagctc

SEQ ID NO: 62 - DNA, 23 bp, Artificial Sequence
  Description of Artificial Sequence: Synthetic primer
ttttttttttttttttttgaagc

SEQ ID NO: 63 - DNA, 51 bp, Artificial Sequence; identical to SEQ ID NO: 34
  Description of Artificial Sequence: Synthetic primer

SEQ ID NO: 64 - DNA, 48 bp, Artificial Sequence; identical to SEQ ID NO: 43
  Description of Artificial Sequence: Synthetic primer

SEQ ID NO: 65 - DNA, 26 bp, Artificial Sequence
  Description of Artificial Sequence: Synthetic primer
ttttttttttttttttttgaagctcc

SEQ ID NO: 66 - DNA, 25 bp, Artificial Sequence
  Description of Artificial Sequence: Synthetic primer
ttttttttttttttttttgaagctc

SEQ ID NO: 67 - DNA, 26 bp, Artificial Sequence
  Description of Artificial Sequence: Synthetic primer
  Description of Combined DNA/RNA Molecule: Synthetic primer
ttutttutttutttttttgaagctcc

SEQ ID NO: 68 - DNA, 25 bp, Artificial Sequence
  Description of Artificial Sequence: Synthetic primer
  Description of Combined DNA/RNA Molecule: Synthetic primer
ttutttutttutttttttgaagctc

SEQ ID NO: 69 - DNA, 23 bp, Artificial Sequence
  Description of Artificial Sequence: Synthetic primer
  Description of Combined DNA/RNA Molecule: Synthetic primer
ttutttutttutttttttgaagc

SEQ ID NO: 70 - DNA, 48 bp, Artificial Sequence
  Description of Artificial Sequence: Synthetic primer
  Description of Combined DNA/RNA Molecule: Synthetic primer
gatcaacgtgtcaccgcctattctattutttutttutttutttgaagc

SEQ ID NO: 71 - DNA, 26 bp, Artificial Sequence
  Description of Artificial Sequence: Synthetic primer
  Description of Combined DNA/RNA Molecule: Synthetic primer
ttttttttttttttttttgaagcucc

SEQ ID NO: 72 - DNA, 26 bp, Artificial Sequence
  Description of Artificial Sequence: Synthetic primer
  Description of Combined DNA/RNA Molecule: Synthetic primer
ttttttttttttttttttgaagcucc

SEQ ID NO: 73 - DNA, 51 bp, Artificial Sequence
  Description of Artificial Sequence: Synthetic primer
  Description of Combined DNA/RNA Molecule: Synthetic primer
gatcaacgtgtcaccgcctattctattttttttttttttttttgaagcucc

SEQ ID NO: 74 - DNA, 51 bp, Artificial Sequence; identical to SEQ ID NO: 73
  Description of Artificial Sequence: Synthetic primer
  Description of Combined DNA/RNA Molecule: Synthetic primer

SEQ ID NO: 75 - DNA, 51 bp, Artificial Sequence
  Description of Artificial Sequence: Synthetic primer
  Description of Combined DNA/RNA Molecule: Synthetic primer
aactgctgcttaaatcttgctacccttttttttttttttttttgaagcucc

SEQ ID NO: 76 - DNA, 51 bp, Artificial Sequence; identical to SEQ ID NO: 75
  Description of Artificial Sequence: Synthetic primer
  Description of Combined DNA/RNA Molecule: Synthetic primer

SEQ ID NO: 77 - DNA, 51 bp, Artificial Sequence; identical to SEQ ID NO: 73
  Description of Artificial Sequence: Synthetic primer
  Description of Combined DNA/RNA Molecule: Synthetic primer

SEQ ID NO: 78 - DNA, 51 bp, Artificial Sequence; identical to SEQ ID NO: 50
  Description of Artificial Sequence: Synthetic primer

SEQ ID NO: 79 - DNA, 48 bp, Artificial Sequence; identical to SEQ ID NO: 51
  Description of Artificial Sequence: Synthetic primer

SEQ ID NO: 80 - DNA, 26 bp, Artificial Sequence
  Description of Artificial Sequence: Synthetic primer
ttttttttttttttttttgtagctcc

SEQ ID NO: 81 - DNA, 23 bp, Artificial Sequence
  Description of Artificial Sequence: Synthetic primer
ttttttttttttttttttgtagc

SEQ ID NO: 82 - DNA, 25 bp, Artificial Sequence
  Description of Artificial Sequence: Synthetic primer
ttttttttttttttttttgtagctc

SEQ ID NO: 83 - DNA, 51 bp, Artificial Sequence
  Description of Artificial Sequence: Synthetic primer
gatcaacgtgtcaccgcctattctatttttttttttttttttttttttttg

SEQ ID NO: 84 - DNA, 51 bp, Artificial Sequence
  Description of Artificial Sequence: Synthetic primer
  Description of Combined DNA/RNA Molecule: Synthetic primer
gatcaacgtgtcaccgcctattctatttttttttuuutttuuutttuuutg

SEQ ID NO: 85 - DNA, 48 bp, Artificial Sequence
  Description of Artificial Sequence: Synthetic primer
  Description of Combined DNA/RNA Molecule: Synthetic primer
gatcaacgtgtcaccgcctattctatttttttttttttuuuttgaagc

SEQ ID NO: 86 - DNA, 51 bp, Artificial Sequence
  Description of Artificial Sequence: Synthetic primer
  Description of Combined DNA/RNA Molecule: Synthetic primer
gatcaacgtgtcaccgcctattctatttttttuuutttuuuttgaagctcc

SEQ ID NO: 87 - DNA, 26 bp, Artificial Sequence
  Description of Artificial Sequence: Synthetic primer
  Description of Combined DNA/RNA Molecule: Synthetic primer
tttttttttttttuuuttgaagctcc

SEQ ID NO: 88 - DNA, 48 bp, Artificial Sequence
  Description of Artificial Sequence: Synthetic primer
  Description of Combined DNA/RNA Molecule: Synthetic primer
gatcaacgtgtcaccgcctattctattttttutttutttutttgaagc

SEQ ID NO: 89 - DNA, 51 bp, Artificial Sequence
  Description of Artificial Sequence: Synthetic primer
  Description of Combined DNA/RNA Molecule: Synthetic primer
gatcaacgtgtcaccgcctattctattttttutttutttutttgaagctcc

SEQ ID NO: 90 - DNA, 26 bp, Artificial Sequence
  Description of Artificial Sequence: Synthetic primer
  Description of Combined DNA/RNA Molecule: Synthetic primer
ttttttutttutttutttgaagctcc

SEQ ID NO: 91 - DNA, 26 bp, Artificial Sequence
  Description of Artificial Sequence: Synthetic primer
ttttttttttttttttttgaagctcc

SEQ ID NO: 92 - DNA, 48 bp, Artificial Sequence
  Description of Artificial Sequence: Synthetic primer
  Description of Combined DNA/RNA Molecule: Synthetic primer
gatcaacgtgtcaccgcctattctattutututuuutttututgaagc

SEQ ID NO: 93 - DNA, 26 bp, Artificial Sequence
  Description of Artificial Sequence: Synthetic primer
  Description of Combined DNA/RNA Molecule: Synthetic primer
ttuuutttuuutttuuutgtagctcc

SEQ ID NO: 94 - DNA, 48 bp, Artificial Sequence
  Description of Artificial Sequence: Synthetic primer
  Description of Combined DNA/RNA Molecule: Synthetic primer
gatcaacgtgtcaccgcctattctattutututuuutttututgtagc

SEQ ID NO: 95 - DNA, 47 bp, Artificial Sequence
  Description of Artificial Sequence: Synthetic primer
gatcaacgtgtcaccgcctattctatttttttttttttttttgaagc

SEQ ID NO: 96 - DNA, 47 bp, Artificial Sequence
  Description of Artificial Sequence: Synthetic primer
gatcaacgtgtcaccgcctattctatttttttttttttttttgtagc

SEQ ID NO: 97 - DNA, 48 bp, Artificial Sequence
  Description of Artificial Sequence: Synthetic primer
  Description of Combined DNA/RNA Molecule: Synthetic primer
gatcaacgtgtcaccgcctattctaututututttutttuuutgaagc

SEQ ID NO: 98 - DNA, 48 bp, Artificial Sequence
  Description of Artificial Sequence: Synthetic primer
  Description of Combined DNA/RNA Molecule: Synthetic primer
gatcaacgtgtcaccgcctattctaututututttutttuuutgtagc

SEQ ID NO: 99 - DNA, 47 bp, Artificial Sequence
  Description of Artificial Sequence: Synthetic primer
  Description of Combined DNA/RNA Molecule: Synthetic primer
gatcaacgtgtcaccgcctattctatutttutttutttututgaagc

SEQ ID NO: 100 - DNA, 47 bp, Artificial Sequence
  Description of Artificial Sequence: Synthetic primer
  Description of Combined DNA/RNA Molecule: Synthetic primer
gatcaacgtgtcaccgcctattctatutttutttutttututgtagc

SEQ ID NO: 101 - DNA, 48 bp, Artificial Sequence; identical to SEQ ID NO: 92
  Description of Artificial Sequence: Synthetic primer
  Description of Combined DNA/RNA Molecule: Synthetic primer

SEQ ID NO: 102 - DNA, 48 bp, Artificial Sequence; identical to SEQ ID NO: 94
  Description of Artificial Sequence: Synthetic primer
  Description of Combined DNA/RNA Molecule: Synthetic primer

SEQ ID NO: 103 - DNA, 47 bp, Artificial Sequence; identical to SEQ ID NO: 95
  Description of Artificial Sequence: Synthetic primer

SEQ ID NO: 104 - DNA, 47 bp, Artificial Sequence; identical to SEQ ID NO: 96
  Description of Artificial Sequence: Synthetic primer

SEQ ID NO: 105 - DNA, 42 bp, Artificial Sequence
  Description of Artificial Sequence: Synthetic primer
  Description of Combined DNA/RNA Molecule: Synthetic primer
cgtgtcaccgcctattctattutututuuutttututgaagc

SEQ ID NO: 106 - DNA, 42 bp, Artificial Sequence
  Description of Artificial Sequence: Synthetic primer
  Description of Combined DNA/RNA Molecule: Synthetic primer
cgtgtcaccgcctattctattutututuuutttututgtagc

SEQ ID NO: 107 - DNA, 42 bp, Artificial Sequence
  Description of Artificial Sequence: Synthetic primer
  Description of Combined DNA/RNA Molecule: Synthetic primer
gatcaacgtgtcaccgcctttutututuuutttututgaagc

SEQ ID NO: 108 - DNA, 42 bp, Artificial Sequence
  Description of Artificial Sequence: Synthetic primer
  Description of Combined DNA/RNA Molecule: Synthetic primer
gatcaacgtgtcaccgcctttutututuuutttututgtagc

SEQ ID NO: 109 - DNA, 45 bp, Artificial Sequence
  Description of Artificial Sequence: Synthetic primer
  Description of Combined DNA/RNA Molecule: Synthetic primer
cgtgtcaccgcctattctattutututuuutttututgaagctcc

SEQ ID NO: 110 - DNA, 45 bp, Artificial Sequence
  Description of Artificial Sequence: Synthetic primer
  Description of Combined DNA/RNA Molecule: Synthetic primer
cgtgtcaccgcctattctattutututuuutttututgtagctcc

SEQ ID NO: 111 - DNA, 45 bp, Artificial Sequence
  Description of Artificial Sequence: Synthetic primer
  Description of Combined DNA/RNA Molecule: Synthetic primer
gatcaacgtgtcaccgcctttutututuuutttututgaagctcc

SEQ ID NO: 112 - DNA, 45 bp, Artificial Sequence
  Description of Artificial Sequence: Synthetic primer
  Description of Combined DNA/RNA Molecule: Synthetic primer
gatcaacgtgtcaccgcctttutututuuutttututgtagctcc

SEQ ID NO: 113 - DNA, 42 bp, Artificial Sequence; identical to SEQ ID NO: 106
  Description of Artificial Sequence: Synthetic primer
  Description of Combined DNA/RNA Molecule: Synthetic primer

SEQ ID NO: 114 - DNA, 48 bp, Artificial Sequence; identical to SEQ ID NO: 94
  Description of Artificial Sequence: Synthetic primer
  Description of Combined DNA/RNA Molecule: Synthetic primer

SEQ ID NO: 115 - DNA, 48 bp, Artificial Sequence
  Description of Artificial Sequence: Synthetic primer
  Description of Combined DNA/RNA Molecule: Synthetic primer
gatcaacgtgtcaccgcctattctautututuuutttututgaagctc

SEQ ID NO: 116 - DNA, 48 bp, Artificial Sequence
  Description of Artificial Sequence: Synthetic primer
  Description of Combined DNA/RNA Molecule: Synthetic primer
gatcaacgtgtcaccgcctattctautututuuutttututgtagctc

SEQ ID NO: 117 - DNA, 48 bp, Artificial Sequence
  Description of Artificial Sequence: Synthetic primer
  Description of Combined DNA/RNA Molecule: Synthetic primer
gatcaacgtgtcaccgcctattctatutututuuutttututgtagct

SEQ ID NO: 118 - DNA, 48 bp, Artificial Sequence
  Description of Artificial Sequence: Synthetic primer
  Description of Combined DNA/RNA Molecule: Synthetic primer
  modified_base (47)..(47): Inosine
gatcaacgtgtcaccgcctattctattutututuuutttututgtanc

SEQ ID NO: 119 - DNA, 46 bp, Artificial Sequence
  Description of Artificial Sequence: Synthetic primer
  Description of Combined DNA/RNA Molecule: Synthetic primer
gatcaacgtgtcaccgcctttutututuuutttututgtagctcca

SEQ ID NO: 120 - DNA, 46 bp, Artificial Sequence
  Description of Artificial Sequence: Synthetic primer
  Description of Combined DNA/RNA Molecule: Synthetic primer
gatcaacgtgtcaccgcctttutututuuutttututgaagctcca

SEQ ID NO: 121 - DNA, 47 bp, Artificial Sequence
  Description of Artificial Sequence: Synthetic primer
  Description of Combined DNA/RNA Molecule: Synthetic primer
gatcaacgtgtcaccgcctttutututuuutttututgtagctccaa

SEQ ID NO: 122 - DNA, 47 bp, Artificial Sequence
  Description of Artificial Sequence: Synthetic primer
  Description of Combined DNA/RNA Molecule: Synthetic primer
gatcaacgtgtcaccgcctttutututuuutttututgaagctccaa

SEQ ID NO: 123 - DNA, 48 bp, Artificial Sequence
  Description of Artificial Sequence: Synthetic primer
  Description of Combined DNA/RNA Molecule: Synthetic primer
gatcaacgtgtcaccgcctttutututuuutttututgtagctccaaa

SEQ ID NO: 124 - DNA, 51 bp, Artificial Sequence
  Description of Artificial Sequence: Synthetic primer
  Description of Combined DNA/RNA Molecule: Synthetic primer
gatcaacgtgtcaccgcctttutututuuutttututgtagctccaaattc

SEQ ID NO: 125 - DNA, 51 bp, Artificial Sequence
  Description of Artificial Sequence: Synthetic primer
  Description of Combined DNA/RNA Molecule: Synthetic primer
gatcaacgtgtcaccgcctttutututuuutttututgaagctccaaattc

SEQ ID NO: 126 - DNA, 45 bp, Artificial Sequence
  Description of Artificial Sequence: Synthetic primer
  Description of Combined DNA/RNA Molecule: Synthetic primer
  modified_base (41)..(41): Inosine
gatcaacgtgtcaccgcctttutututuuutttututgtanctcc

SEQ ID NO: 127 - DNA, 45 bp, Artificial Sequence; identical to SEQ ID NO: 112
  Description of Artificial Sequence: Synthetic primer
  Description of Combined DNA/RNA Molecule: Synthetic primer

SEQ ID NO: 128 - DNA, 45 bp, Artificial Sequence; identical to SEQ ID NO: 112
  Description of Artificial Sequence: Synthetic primer
  Description of Combined DNA/RNA Molecule: Synthetic primer

SEQ ID NO: 129 - DNA, 45 bp, Artificial Sequence; identical to SEQ ID NO: 112
  Description of Artificial Sequence: Synthetic primer
  Description of Combined DNA/RNA Molecule: Synthetic primer

SEQ ID NO: 130 - DNA, 45 bp, Artificial Sequence; identical to SEQ ID NO: 112
  Description of Artificial Sequence: Synthetic primer
  Description of Combined DNA/RNA Molecule: Synthetic primer

SEQ ID NO: 131 - DNA, 45 bp, Artificial Sequence
  Description of Artificial Sequence: Synthetic primer
  Description of Combined DNA/RNA Molecule: Synthetic primer
  modified_base (38)..(38): Inosine
  modified_base (41)..(41): Inosine
gatcaacgtgtcaccgcctttutututuuutttututntanctcc

SEQ ID NO: 132 - DNA, 41 bp, Artificial Sequence
  Description of Artificial Sequence: Synthetic primer
gatcaacgtgtcaccgccttttttttttttttttttgtagc

SEQ ID NO: 133 - DNA, 43 bp, Artificial Sequence
  Description of Artificial Sequence: Synthetic primer
gatcaacgtgtcaccgccttttttttttttttttttgtagctc

SEQ ID NO: 134 - DNA, 43 bp, Artificial Sequence
  Description of Artificial Sequence: Synthetic primer
gatcaacgtgtcaccgccttttttttttttttttttgaagctc

SEQ ID NO: 135 - DNA, 44 bp, Artificial Sequence
  Description of Artificial Sequence: Synthetic primer
gatcaacgtgtcaccgccttttttttttttttttttgtagctcc

SEQ ID NO: 136 - DNA, 44 bp, Artificial Sequence
  Description of Artificial Sequence: Synthetic primer
gatcaacgtgtcaccgccttttttttttttttttttgaagctcc

SEQ ID NO: 137 - DNA, 45 bp, Artificial Sequence
  Description of Artificial Sequence: Synthetic primer
gatcaacgtgtcaccgccttttttttttttttttttgtagctcca

SEQ ID NO: 138 - DNA, 45 bp, Artificial Sequence
  Description of Artificial Sequence: Synthetic primer
gatcaacgtgtcaccgccttttttttttttttttttgaagctcca

SEQ ID NO: 139 - DNA, 46 bp, Artificial Sequence
  Description of Artificial Sequence: Synthetic primer
gatcaacgtgtcaccgccttttttttttttttttttgtagctccaa

SEQ ID NO: 140 - DNA, 46 bp, Artificial Sequence
  Description of Artificial Sequence: Synthetic primer
gatcaacgtgtcaccgccttttttttttttttttttgaagctccaa

SEQ ID NO: 141 - DNA, 38 bp, Artificial Sequence
  Description of Artificial Sequence: Synthetic primer
  Description of Combined DNA/RNA Molecule: Synthetic primer
gatcaacgtgtcaccgccuuuuuuuuuuuugaagctcc

SEQ ID NO: 142 - DNA, 38 bp, Artificial Sequence
  Description of Artificial Sequence: Synthetic primer
  Description of Combined DNA/RNA Molecule: Synthetic primer
gatcaacgtgtcaccgccuuuuuuuuuuuugtagctcc

SEQ ID NO: 143 - DNA, 38 bp, Artificial Sequence
  Description of Artificial Sequence: Synthetic primer
  Description of Combined DNA/RNA Molecule: Synthetic primer
gatcaacgtgtcaccgccuuuuuuuuuuuugacgctcc

SEQ ID NO: 144 - DNA, 38 bp, Artificial Sequence
  Description of Artificial Sequence: Synthetic primer
  Description of Combined DNA/RNA Molecule: Synthetic primer
gatcaacgtgtcaccgccuuuuuuuuuuuugaagcgcc

SEQ ID NO: 145 - DNA, 38 bp, Artificial Sequence
  Description of Artificial Sequence: Synthetic primer
  Description of Combined DNA/RNA Molecule: Synthetic primer
gatcaacgtgtcaccgccuuuuuuuuuuuugacgcgcc

SEQ ID NO: 146 - DNA, 38 bp, Artificial Sequence
  Description of Artificial Sequence: Synthetic primer
  Description of Combined DNA/RNA Molecule: Synthetic primer
gatcaacgtgtcaccgccuuuuuuuuuuuugcagcgcc

SEQ ID NO: 147 - DNA, 45 bp, Artificial Sequence
  Description of Artificial Sequence: Synthetic primer
  Description of Combined DNA/RNA Molecule: Synthetic primer
gatcaacgtgtcaccgcctttutututuuutttututgacgctcc

SEQ ID NO: 148 - DNA, 45 bp, Artificial Sequence
  Description of Artificial Sequence: Synthetic primer
  Description of Combined DNA/RNA Molecule: Synthetic primer
gatcaacgtgtcaccgcctttutututuuutttututgaagcgcc

SEQ ID NO: 149 - DNA, 45 bp, Artificial Sequence
  Description of Artificial Sequence: Synthetic primer
  Description of Combined DNA/RNA Molecule: Synthetic primer
gatcaacgtgtcaccgcctttutututuuutttututgacgcgcc

SEQ ID NO: 150 - DNA, 45 bp, Artificial Sequence
  Description of Artificial Sequence: Synthetic primer
  Description of Combined DNA/RNA Molecule: Synthetic primer
gatcaacgtgtcaccgcctttutututuuutttututgcagcgcc

SEQ ID NO: 151 - DNA, 49 bp, Artificial Sequence
  Description of Artificial Sequence: Synthetic primer
gatcaacgtgtcaccgcctattctatttttttttttttttttgtagctc

SEQ ID NO: 152 - DNA, 49 bp, Artificial Sequence
  Description of Artificial Sequence: Synthetic primer
gatcaacgtgtcaccgcctattctatttttttttttttttttgaagctc

SEQ ID NO: 153 - DNA, 49 bp, Artificial Sequence
  Description of Artificial Sequence: Synthetic primer
gatcaacgtgtcaccgcctattctattttttttttttttttgtagctcc

SEQ ID NO: 154 - DNA, 49 bp, Artificial Sequence
  Description of Artificial Sequence: Synthetic primer
gatcaacgtgtcaccgcctattctattttttttttttttttgaagctcc

SEQ ID NO: 155 - DNA, 49 bp, Artificial Sequence
  Description of Artificial Sequence: Synthetic primer
gatcaacgtgtcaccgcctattctatttttttttttttttgtagctcca

SEQ ID NO: 156 - DNA, 49 bp, Artificial Sequence
  Description of Artificial Sequence: Synthetic primer
gatcaacgtgtcaccgcctattctatttttttttttttttgaagctcca

SEQ ID NO: 157 - DNA, 49 bp, Artificial Sequence
  Description of Artificial Sequence: Synthetic primer
gatcaacgtgtcaccgcctattctattttttttttttttgtagctccaa

SEQ ID NO: 158 - DNA, 49 bp, Artificial Sequence
  Description of Artificial Sequence: Synthetic primer
gatcaacgtgtcaccgcctattctattttttttttttttgaagctccaa

SEQ ID NO: 159 - DNA, 49 bp, Artificial Sequence; identical to SEQ ID NO: 151
  Description of Artificial Sequence: Synthetic primer

SEQ ID NO: 160 - DNA, 49 bp, Artificial Sequence; identical to SEQ ID NO: 152
  Description of Artificial Sequence: Synthetic primer

SEQ ID NO: 161 - DNA, 39 bp, Artificial Sequence
  Description of Artificial Sequence: Synthetic primer
  Description of Combined DNA/RNA Molecule: Synthetic primer
gatcaacgtgtcaccgccuuuuuuuuuuuugaagctcca

SEQ ID NO: 162 - DNA, 39 bp, Artificial Sequence
  Description of Artificial Sequence: Synthetic primer
  Description of Combined DNA/RNA Molecule: Synthetic primer
gatcaacgtgtcaccgccuuuuuuuuuuuugtagctcca

SEQ ID NO: 163 - DNA, 40 bp, Artificial Sequence
  Description of Artificial Sequence: Synthetic primer
  Description of Combined DNA/RNA Molecule: Synthetic primer
gatcaacgtgtcaccgccuuuuuuuuuuuugaagctccaa

SEQ ID NO: 164 - DNA, 40 bp, Artificial Sequence
  Description of Artificial Sequence: Synthetic primer
  Description of Combined DNA/RNA Molecule: Synthetic primer
gatcaacgtgtcaccgccuuuuuuuuuuuugtagctccaa

SEQ ID NO: 165 - DNA, 46 bp, Artificial Sequence; identical to SEQ ID NO: 119
  Description of Artificial Sequence: Synthetic primer
  Description of Combined DNA/RNA Molecule: Synthetic primer

SEQ ID NO: 166 - DNA, 47 bp, Artificial Sequence; identical to SEQ ID NO: 121
  Description of Artificial Sequence: Synthetic primer
  Description of Combined DNA/RNA Molecule: Synthetic primer

SEQ ID NO: 167 - DNA, 48 bp, Artificial Sequence; identical to SEQ ID NO: 123
  Description of Artificial Sequence: Synthetic primer
  Description of Combined DNA/RNA Molecule: Synthetic primer

SEQ ID NO: 168 - DNA, 50 bp, Artificial Sequence
  Description of Artificial Sequence: Synthetic primer
gatcaacgtgtcaccgcctattctatttttttttttttttttgtagctcc

SEQ ID NO: 169 - DNA, 50 bp, Artificial Sequence
  Description of Artificial Sequence: Synthetic primer
gatcaacgtgtcaccgcctattctatttttttttttttttttgaagctcc

SEQ ID NO: 170 - DNA, 50 bp, Artificial Sequence
  Description of Artificial Sequence: Synthetic primer
gatcaacgtgtcaccgcctattctattttttttttttttttgtagctcca

SEQ ID NO: 171 - DNA, 50 bp, Artificial Sequence
  Description of Artificial Sequence: Synthetic primer
gatcaacgtgtcaccgcctattctattttttttttttttttgaagctcca

SEQ ID NO: 172 - DNA, 45 bp, Artificial Sequence
  Description of Artificial Sequence: Synthetic primer
gatcaacgtgtcaccgcctattctattttttttttttgtagctcc

SEQ ID NO: 173 - DNA, 45 bp, Artificial Sequence; identical to SEQ ID NO: 48
  Description of Artificial Sequence: Synthetic primer

SEQ ID NO: 174 - DNA, 46 bp, Artificial Sequence
  Description of Artificial Sequence: Synthetic primer
gatcaacgtgtcaccgcctattctattttttttttttgtagctcca

SEQ ID NO: 175 - DNA, 46 bp, Artificial Sequence
  Description of Artificial Sequence: Synthetic primer
gatcaacgtgtcaccgcctattctattttttttttttgaagctcca

SEQ ID NO: 176 - DNA, 44 bp, Artificial Sequence; identical to SEQ ID NO: 135
  Description of Artificial Sequence: Synthetic primer

SEQ ID NO: 177 - DNA, 44 bp, Artificial Sequence; identical to SEQ ID NO: 136
  Description of Artificial Sequence: Synthetic primer

SEQ ID NO: 178 - DNA, 45 bp, Artificial Sequence; identical to SEQ ID NO: 137
  Description of Artificial Sequence: Synthetic primer

SEQ ID NO: 179 - DNA, 45 bp, Artificial Sequence; identical to SEQ ID NO: 138
  Description of Artificial Sequence: Synthetic primer

SEQ ID NO: 180 - DNA, 47 bp, Artificial Sequence
  Description of Artificial Sequence: Synthetic primer
gatcaacgtgtcaccgcctattctattttttttttttgtagctccaa

SEQ ID NO: 181 - DNA, 47 bp, Artificial Sequence
  Description of Artificial Sequence: Synthetic primer
gatcaacgtgtcaccgcctattctattttttttttttgaagctccaa

SEQ ID NO: 182 - DNA, 46 bp, Artificial Sequence; identical to SEQ ID NO: 139
  Description of Artificial Sequence: Synthetic primer

SEQ ID NO: 183 - DNA, 46 bp, Artificial Sequence; identical to SEQ ID NO: 140
  Description of Artificial Sequence: Synthetic primer

SEQ ID NO: 184 - DNA, 47 bp, Artificial Sequence; identical to SEQ ID NO: 96
  Description of Artificial Sequence: Synthetic primer

SEQ ID NO: 185 - DNA, 37 bp, Artificial Sequence
  Description of Artificial Sequence: Synthetic primer
  Description of Combined DNA/RNA Molecule: Synthetic primer
gatcaacgtgtcaccgccuuuuuuuuuuuugaagctc

SEQ ID NO: 186 - DNA, 37 bp, Artificial Sequence
  Description of Artificial Sequence: Synthetic primer
  Description of Combined DNA/RNA Molecule: Synthetic primer
gatcaacgtgtcaccgccuuuuuuuuuuuugtagctc

SEQ ID NO: 187 - DNA, 44 bp, Artificial Sequence
  Description of Artificial Sequence: Synthetic primer
gatcaacgtgtcaccgcctattctattttttttttttgtagctc

SEQ ID NO: 188 - DNA, 44 bp, Artificial Sequence
  Description of Artificial Sequence: Synthetic primer
gatcaacgtgtcaccgcctattctattttttttttttgaagctc

SEQ ID NO: 189 - DNA, 43 bp, Artificial Sequence; identical to SEQ ID NO: 133
  Description of Artificial Sequence: Synthetic primer

SEQ ID NO: 190 - DNA, 43 bp, Artificial Sequence; identical to SEQ ID NO: 134
  Description of Artificial Sequence: Synthetic primer

SEQ ID NO: 191 - DNA, 23 bp, Artificial Sequence
  Description of Artificial Sequence: Synthetic oligonucleotide
aactccacagaagctccaaattc

SEQ ID NO: 192 - DNA, 28 bp, Artificial Sequence
  Description of Artificial Sequence: Synthetic oligonucleotide
agagtaactccacagaagctccaaattc

SEQ ID NO: 193 - DNA, 22 bp, Artificial Sequence
  Description of Artificial Sequence: Synthetic oligonucleotide
gagagtaactccacagaagctc

SEQ ID NO: 194 - DNA, 20 bp, Artificial Sequence
  Description of Artificial Sequence: Synthetic oligonucleotide
gagagtaactccacagaagc

SEQ ID NO: 195 - DNA, 20 bp, Artificial Sequence
  Description of Artificial Sequence: Synthetic oligonucleotide
gagagtaactccacagaagc

SEQ ID NO: 196 - DNA, 34 bp, Artificial Sequence; identical to SEQ ID NO: 6
  Description of Artificial Sequence: Synthetic oligonucleotide
  modified_base (14)..(14): a, c, t, g, unknown or other

SEQ ID NO: 197 - DNA, 29 bp, Artificial Sequence
  Description of Artificial Sequence: Synthetic oligonucleotide
  modified_base (9)..(9): a, c, t, g, unknown or other
ggcaaaaangagagtaactccacagaagc

SEQ ID NO: 198 - DNA, 20 bp, Artificial Sequence
  Description of Artificial Sequence: Synthetic oligonucleotide
gagagtaactccacagaagc

SEQ ID NO: 199 - DNA, 28 bp, Artificial Sequence
  Description of Artificial Sequence: Synthetic oligonucleotide
agagtaactccacagaagctccaaattc

SEQ ID NO: 200 - DNA, 28 bp, Artificial Sequence
  Description of Artificial Sequence: Synthetic oligonucleotide
agagtaactccacagaagctccaaattc

SEQ ID NO: 201 - DNA, 29 bp, Artificial Sequence
  Description of Artificial Sequence: Synthetic oligonucleotide
gagagtaactccacagaagctccaaattc

SEQ ID NO: 202 - DNA, 29 bp, Artificial Sequence
  Description of Artificial Sequence: Synthetic oligonucleotide
gagagtaactccacagaagctccaaattc

SEQ ID NO: 203 - DNA, 43 bp, Artificial Sequence; identical to SEQ ID NO: 13
  Description of Artificial Sequence: Synthetic oligonucleotide
  modified_base (14)..(14): a, c, t, g, unknown or other

SEQ ID NO: 204 - DNA, 49 bp, Artificial Sequence; identical to SEQ ID NO: 14
  Description of Artificial Sequence: Synthetic oligonucleotide
  modified_base (14)..(14): a, c, t, g, unknown or other

SEQ ID NO: 205 - DNA, 20 bp, Artificial Sequence
  Description of Artificial Sequence: Synthetic oligonucleotide
gagagtaactccacagaagc

SEQ ID NO: 206 - DNA, 25 bp, Artificial Sequence
  Description of Artificial Sequence: Synthetic oligonucleotide
ttttttttttttttttttgctggtg

SEQ ID NO: 207 - DNA, 28 bp, Artificial Sequence
  Description of Artificial Sequence: Synthetic oligonucleotide
tgtactaggaggctgtaggcataaattg

SEQ ID NO: 208 - DNA, 50 bp, Artificial Sequence; identical to SEQ ID NO: 18
  Description of Artificial Sequence: Synthetic oligonucleotide

SEQ ID NO: 209 - DNA, 50 bp, Artificial Sequence; identical to SEQ ID NO: 19
  Description of Artificial Sequence: Synthetic oligonucleotide

SEQ ID NO: 210 - DNA, 22 bp, Artificial Sequence
  Description of Artificial Sequence: Synthetic oligonucleotide
ttgaggcatacttcaaagactg

SEQ ID NO: 211 - DNA, 35 bp, Artificial Sequence; identical to SEQ ID NO: 21
  Description of Artificial Sequence: Synthetic oligonucleotide
  modified_base (18)..(19): a, c, t, g, unknown or other

SEQ ID NO: 212 - DNA, 23 bp, Artificial Sequence
  Description of Artificial Sequence: Synthetic oligonucleotide
  modified_base (11)..(12): a, c, t, g, unknown or other
ggtgctggtgnncagacccaatt

SEQ ID NO: 213 - DNA, 23 bp, Artificial Sequence
  Description of Artificial Sequence: Synthetic oligonucleotide
actcttggactctcagcaatgtc

SEQ ID NO: 214 - DNA, 23 bp, Artificial Sequence
  Description of Artificial Sequence: Synthetic oligonucleotide
actcttggactctctgtaatgtc

SEQ ID NO: 215 - DNA, 28 bp, Artificial Sequence
  Description of Artificial Sequence: Synthetic oligonucleotide
ttttttttttttttttttgctggtgaac

SEQ ID NO: 216 - DNA, 28 bp, Artificial Sequence
  Description of Artificial Sequence: Synthetic oligonucleotide
ttttttttttttttttttgctggtgcgc

SEQ ID NO: 217 - DNA, 53 bp, Artificial Sequence; identical to SEQ ID NO: 27
  Description of Artificial Sequence: Synthetic oligonucleotide

SEQ ID NO: 218 - DNA, 53 bp, Artificial Sequence; identical to SEQ ID NO: 28
  Description of Artificial Sequence: Synthetic oligonucleotide

SEQ ID NO: 219 - DNA, 53 bp, Artificial Sequence; identical to SEQ ID NO: 29
  Description of Artificial Sequence: Synthetic oligonucleotide

SEQ ID NO: 220 - DNA, 53 bp, Artificial Sequence; identical to SEQ ID NO: 30
  Description of Artificial Sequence: Synthetic oligonucleotide

SEQ ID NO: 221 - DNA, 41 bp, Artificial Sequence; identical to SEQ ID NO: 31
  Description of Artificial Sequence: Synthetic oligonucleotide

SEQ ID NO: 222 - DNA, 41 bp, Artificial Sequence; identical to SEQ ID NO: 32
  Description of Artificial Sequence: Synthetic oligonucleotide

SEQ ID NO: 223 - DNA, 51 bp, Artificial Sequence; identical to SEQ ID NO: 33
  Description of Artificial Sequence: Synthetic oligonucleotide

SEQ ID NO: 224 - DNA, 51 bp, Artificial Sequence; identical to SEQ ID NO: 34
  Description of Artificial Sequence: Synthetic oligonucleotide

SEQ ID NO: 225 - DNA, 51 bp, Artificial Sequence; identical to SEQ ID NO: 35
  Description of Artificial Sequence: Synthetic oligonucleotide

SEQ ID NO: 226 - DNA, 25 bp, Artificial Sequence
  Description of Artificial Sequence: Synthetic oligonucleotide
atagaagagctgtcgtagtctccga

SEQ ID NO: 227 - DNA, 25 bp, Artificial Sequence
  Description of Artificial Sequence: Synthetic oligonucleotide
gatcaacgtgtcaccgcctattcta

SEQ ID NO: 228 - DNA, 25 bp, Artificial Sequence
  Description of Artificial Sequence: Synthetic oligonucleotide
aactgctgcttaaatcttgctaccc

SEQ ID NO: 229 - DNA, 26 bp, Artificial Sequence
  Description of Artificial Sequence: Synthetic oligonucleotide
ttttttttttttttttttgaagctcc

SEQ ID NO: 230 - DNA, 50 bp, Artificial Sequence; identical to SEQ ID NO: 40
  Description of Artificial Sequence: Synthetic oligonucleotide

SEQ ID NO: 231 - DNA, 50 bp, Artificial Sequence; identical to SEQ ID NO: 41
  Description of Artificial Sequence: Synthetic oligonucleotide

SEQ ID NO: 232 - DNA, 25 bp, Artificial Sequence
  Description of Artificial Sequence: Synthetic oligonucleotide
ttttttttttttttttttgaagctc

SEQ ID NO: 233 - DNA, 48 bp, Artificial Sequence; identical to SEQ ID NO: 43
  Description of Artificial Sequence: Synthetic oligonucleotide

SEQ ID NO: 234 - DNA, 48 bp, Artificial Sequence; identical to SEQ ID NO: 44
  Description of Artificial Sequence: Synthetic oligonucleotide

SEQ ID NO: 235 - DNA, 23 bp, Artificial Sequence
  Description of Artificial Sequence: Synthetic oligonucleotide
ttttttttttttttttttgaagc

SEQ ID NO: 236 - DNA, 48 bp, Artificial Sequence; identical to SEQ ID NO: 46
  Description of Artificial Sequence: Synthetic oligonucleotide

SEQ ID NO: 237 - DNA, 48 bp, Artificial Sequence; identical to SEQ ID NO: 47
  Description of Artificial Sequence: Synthetic oligonucleotide

SEQ ID NO: 238 - DNA, 45 bp, Artificial Sequence; identical to SEQ ID NO: 48
  Description of Artificial Sequence: Synthetic oligonucleotide

SEQ ID NO: 239 - DNA, 45 bp, Artificial Sequence; identical to SEQ ID NO: 49
  Description of Artificial Sequence: Synthetic oligonucleotide

SEQ ID NO: 240 - DNA, 51 bp, Artificial Sequence; identical to SEQ ID NO: 50
  Description of Artificial Sequence: Synthetic oligonucleotide

SEQ ID NO: 241 - DNA, 48 bp, Artificial Sequence; identical to SEQ ID NO: 51
  Description of Artificial Sequence: Synthetic oligonucleotide

SEQ ID NO: 242 - DNA, 26 bp, Artificial Sequence
  Description of Artificial Sequence: Synthetic oligonucleotide
ttttttttttttttttttgtagctcc

SEQ ID NO: 243 - DNA, 23 bp, Artificial Sequence
  Description of Artificial Sequence: Synthetic oligonucleotide
ttttttttttttttttttgtagc

SEQ ID NO: 244 - DNA, 26 bp, Artificial Sequence
  Description of Artificial Sequence: Synthetic oligonucleotide
tttttttttttttttttttttttttg

SEQ ID NO: 245 - DNA, 51 bp, Artificial Sequence; identical to SEQ ID NO: 83
  Description of Artificial Sequence: Synthetic oligonucleotide

SEQ ID NO: 246 - DNA, 26 bp, Artificial Sequence
  Description of Artificial Sequence: Synthetic oligonucleotide
ttttttttttttttttttgaagctcc

SEQ ID NO: 247 - DNA, 26 bp, Artificial Sequence
  Description of Artificial Sequence: Synthetic oligonucleotide
ttttttttttttttttttgaagctcc

SEQ ID NO: 248 - DNA, 26 bp, Artificial Sequence
  Description of Artificial Sequence: Synthetic oligonucleotide
ttttttttttttttttttgaagctcc

SEQ ID NO: 249 - DNA, 26 bp, Artificial Sequence
  Description of Artificial Sequence: Synthetic oligonucleotide
ttttttttttttttttttgaagctcc

SEQ ID NO: 250 - DNA, 26 bp, Artificial Sequence
  Description of Artificial Sequence: Synthetic oligonucleotide
ttttttttttttttttttgaagctcc

SEQ ID NO: 251 - DNA, 25 bp, Artificial Sequence
  Description of Artificial Sequence: Synthetic oligonucleotide
ttttttttttttttttttgaagctc

SEQ ID NO: 252 - DNA, 23 bp, Artificial Sequence
  Description of Artificial Sequence: Synthetic oligonucleotide
ttttttttttttttttttgaagc

SEQ ID NO: 253 - DNA, 51 bp, Artificial Sequence; identical to SEQ ID NO: 34
  Description of Artificial Sequence: Synthetic oligonucleotide

SEQ ID NO: 254 - DNA, 48 bp, Artificial Sequence; identical to SEQ ID NO: 43
  Description of Artificial Sequence: Synthetic oligonucleotide

SEQ ID NO: 255 - DNA, 26 bp, Artificial Sequence
  Description of Artificial Sequence: Synthetic oligonucleotide
ttttttttttttttttttgaagctcc

SEQ ID NO: 256 - DNA, 25 bp, Artificial Sequence
  Description of Artificial Sequence: Synthetic oligonucleotide
ttttttttttttttttttgaagctc

SEQ ID NO: 257 - DNA, 26 bp, Artificial Sequence
  Description of Artificial Sequence: Synthetic oligonucleotide
ttttttttttttttttttgaagctcc

SEQ ID NO: 258 - DNA, 25 bp, Artificial Sequence
  Description of Artificial Sequence: Synthetic oligonucleotide
ttttttttttttttttttgaagctc

SEQ ID NO: 259 - DNA, 23 bp, Artificial Sequence
  Description of Artificial Sequence: Synthetic oligonucleotide
ttttttttttttttttttgaagc

SEQ ID NO: 260 - DNA, 48 bp, Artificial Sequence; identical to SEQ ID NO: 43
  Description of Artificial Sequence: Synthetic oligonucleotide

SEQ ID NO: 261 - DNA, 26 bp, Artificial Sequence
  Description of Artificial Sequence: Synthetic oligonucleotide
ttttttttttttttttttgaagctcc

SEQ ID NO: 262 - DNA, 26 bp, Artificial Sequence
  Description of Artificial Sequence: Synthetic oligonucleotide
ttttttttttttttttttgaagctcc

SEQ ID NO: 263 - DNA, 51 bp, Artificial Sequence; identical to SEQ ID NO: 34
  Description of Artificial Sequence: Synthetic oligonucleotide

SEQ ID NO: 264 - DNA, 51 bp, Artificial Sequence; identical to SEQ ID NO: 34
  Description of Artificial Sequence: Synthetic oligonucleotide

SEQ ID NO: 265 - DNA, 51 bp, Artificial Sequence; identical to SEQ ID NO: 35
  Description of Artificial Sequence: Synthetic oligonucleotide

SEQ ID NO: 266 - DNA, 51 bp, Artificial Sequence; identical to SEQ ID NO: 35
  Description of Artificial Sequence: Synthetic oligonucleotide

SEQ ID NO: 267 - DNA, 51 bp, Artificial Sequence; identical to SEQ ID NO: 34
  Description of Artificial Sequence: Synthetic oligonucleotide

SEQ ID NO: 268 - DNA, 51 bp, Artificial Sequence; identical to SEQ ID NO: 50
  Description of Artificial Sequence: Synthetic oligonucleotide

SEQ ID NO: 269 - DNA, 48 bp, Artificial Sequence; identical to SEQ ID NO: 51
  Description of Artificial Sequence: Synthetic oligonucleotide

SEQ ID NO: 270 - DNA, 26 bp, Artificial Sequence
  Description of Artificial Sequence: Synthetic oligonucleotide
ttttttttttttttttttgtagctcc

SEQ ID NO: 271 - DNA, 23 bp, Artificial Sequence
  Description of Artificial Sequence: Synthetic oligonucleotide
ttttttttttttttttttgtagc

SEQ ID NO: 272 - DNA, 25 bp, Artificial Sequence
  Description of Artificial Sequence: Synthetic oligonucleotide
ttttttttttttttttttgtagctc

SEQ ID NO: 273 - DNA, 51 bp, Artificial Sequence; identical to SEQ ID NO: 83
  Description of Artificial Sequence: Synthetic oligonucleotide

SEQ ID NO: 274 - DNA, 51 bp, Artificial Sequence; identical to SEQ ID NO: 83
  Description of Artificial Sequence: Synthetic oligonucleotide

SEQ ID NO: 275 - DNA, 48 bp, Artificial Sequence; identical to SEQ ID NO: 43
  Description of Artificial Sequence: Synthetic oligonucleotide

SEQ ID NO: 276 - DNA, 51 bp, Artificial Sequence; identical to SEQ ID NO: 34
  Description of Artificial Sequence: Synthetic oligonucleotide

SEQ ID NO: 277 - DNA, 26 bp, Artificial Sequence
  Description of Artificial Sequence: Synthetic oligonucleotide
ttttttttttttttttttgaagctcc

SEQ ID NO: 278 - DNA, 48 bp, Artificial Sequence; identical to SEQ ID NO: 43
  Description of Artificial Sequence: Synthetic oligonucleotide

SEQ ID NO: 279 - DNA, 51 bp, Artificial Sequence; identical to SEQ ID NO: 34
  Description of Artificial Sequence: Synthetic oligonucleotide

SEQ ID NO: 280 - DNA, 26 bp, Artificial Sequence
  Description of Artificial Sequence: Synthetic oligonucleotide
ttttttttttttttttttgaagctcc

SEQ ID NO: 281 - DNA, 26 bp, Artificial Sequence
  Description of Artificial Sequence: Synthetic oligonucleotide
ttttttttttttttttttgaagctcc

SEQ ID NO: 282 - DNA, 48 bp, Artificial Sequence; identical to SEQ ID NO: 43
  Description of Artificial Sequence: Synthetic oligonucleotide

SEQ ID NO: 283 - DNA, 26 bp, Artificial Sequence
  Description of Artificial Sequence: Synthetic oligonucleotide
ttttttttttttttttttgtagctcc

SEQ ID NO: 284 - DNA, 48 bp, Artificial Sequence; identical to SEQ ID NO: 51
  Description of Artificial Sequence: Synthetic oligonucleotide

SEQ ID NO: 285 - DNA, 47 bp, Artificial Sequence; identical to SEQ ID NO: 95
  Description of Artificial Sequence: Synthetic oligonucleotide

SEQ ID NO: 286 - DNA, 47 bp, Artificial Sequence; identical to SEQ ID NO: 96
  Description of Artificial Sequence: Synthetic oligonucleotide

SEQ ID NO: 287 - DNA, 48 bp, Artificial Sequence; identical to SEQ ID NO: 43
  Description of Artificial Sequence: Synthetic oligonucleotide

SEQ ID NO: 288 - DNA, 48 bp, Artificial Sequence; identical to SEQ ID NO: 51
  Description of Artificial Sequence: Synthetic oligonucleotide

SEQ ID NO: 289 - DNA, 47 bp, Artificial Sequence; identical to SEQ ID NO: 95
  Description of Artificial Sequence: Synthetic oligonucleotide

SEQ ID NO: 290 - DNA, 47 bp, Artificial Sequence; identical to SEQ ID NO: 96
  Description of Artificial Sequence: Synthetic oligonucleotide

SEQ ID NO: 291 - DNA, 48 bp, Artificial Sequence; identical to SEQ ID NO: 43
  Description of Artificial Sequence: Synthetic oligonucleotide

SEQ ID NO: 292 - DNA, 48 bp, Artificial Sequence; identical to SEQ ID NO: 51
  Description of Artificial Sequence: Synthetic oligonucleotide

SEQ ID NO: 293 - DNA, 47 bp, Artificial Sequence; identical to SEQ ID NO: 95
  Description of Artificial Sequence: Synthetic oligonucleotide

SEQ ID NO: 294 - DNA, 47 bp, Artificial Sequence; identical to SEQ ID NO: 96
  Description of Artificial Sequence: Synthetic oligonucleotide

SEQ ID NO: 295 - DNA, 42 bp, Artificial Sequence
  Description of Artificial Sequence: Synthetic oligonucleotide
cgtgtcaccgcctattctattttttttttttttttttgaagc

SEQ ID NO: 296 - DNA, 42 bp, Artificial Sequence
  Description of Artificial Sequence: Synthetic oligonucleotide
cgtgtcaccgcctattctattttttttttttttttttgtagc

SEQ ID NO: 297 - DNA, 42 bp, Artificial Sequence
  Description of Artificial Sequence: Synthetic oligonucleotide
gatcaacgtgtcaccgcctttttttttttttttttttgaagc

SEQ ID NO: 298 - DNA, 42 bp, Artificial Sequence
  Description of Artificial Sequence: Synthetic oligonucleotide
gatcaacgtgtcaccgcctttttttttttttttttttgtagc

SEQ ID NO: 299 - DNA, 45 bp, Artificial Sequence
  Description of Artificial Sequence: Synthetic oligonucleotide
cgtgtcaccgcctattctattttttttttttttttttgaagctcc

SEQ ID NO: 300 - DNA, 45 bp, Artificial Sequence
  Description of Artificial Sequence: Synthetic oligonucleotide
cgtgtcaccgcctattctattttttttttttttttttgtagctcc

SEQ ID NO: 301 - DNA, 45 bp, Artificial Sequence
  Description of Artificial Sequence: Synthetic oligonucleotide
gatcaacgtgtcaccgcctttttttttttttttttttgaagctcc

SEQ ID NO: 302 - DNA, 45 bp, Artificial Sequence
  Description of Artificial Sequence: Synthetic oligonucleotide
gatcaacgtgtcaccgcctttttttttttttttttttgtagctcc

SEQ ID NO: 303 - DNA, 42 bp, Artificial Sequence; identical to SEQ ID NO: 296
  Description of Artificial Sequence: Synthetic oligonucleotide

SEQ ID NO: 304 - DNA, 48 bp, Artificial Sequence; identical to SEQ ID NO: 51
  Description of Artificial Sequence: Synthetic oligonucleotide

SEQ ID NO: 305 - DNA, 48 bp, Artificial Sequence
  Description of Artificial Sequence: Synthetic oligonucleotide
gatcaacgtgtcaccgcctattctattttttttttttttttgaagctc

SEQ ID NO: 306 - DNA, 48 bp, Artificial Sequence
  Description of Artificial Sequence: Synthetic oligonucleotide
gatcaacgtgtcaccgcctattctattttttttttttttttgtagctc

SEQ ID NO: 307 - DNA, 48 bp, Artificial Sequence
  Description of Artificial Sequence: Synthetic oligonucleotide
gatcaacgtgtcaccgcctattctatttttttttttttttttgtagct

SEQ ID NO: 308 - DNA, 48 bp, Artificial Sequence; identical to SEQ ID NO: 51
  Description of Artificial Sequence: Synthetic oligonucleotide

SEQ ID NO: 309 - DNA, 46 bp, Artificial Sequence
  Description of Artificial Sequence: Synthetic oligonucleotide
gatcaacgtgtcaccgcctttttttttttttttttttgtagctcca

SEQ ID NO: 310 - DNA, 46 bp, Artificial Sequence
  Description of Artificial Sequence: Synthetic oligonucleotide
gatcaacgtgtcaccgcctttttttttttttttttttgaagctcca

SEQ ID NO: 311 - DNA, 47 bp, Artificial Sequence
  Description of Artificial Sequence: Synthetic oligonucleotide
gatcaacgtgtcaccgcctttttttttttttttttttgtagctccaa

SEQ ID NO: 312 - DNA, 47 bp, Artificial Sequence
  Description of Artificial Sequence: Synthetic oligonucleotide
gatcaacgtgtcaccgcctttttttttttttttttttgaagctccaa

SEQ ID NO: 313 - DNA, 48 bp, Artificial Sequence
  Description of Artificial Sequence: Synthetic oligonucleotide
gatcaacgtgtcaccgcctttttttttttttttttttgtagctccaaa

SEQ ID NO: 314 - DNA, 51 bp, Artificial Sequence
  Description of Artificial Sequence: Synthetic oligonucleotide
gatcaacgtgtcaccgcctttttttttttttttttttgtagctccaaattc

SEQ ID NO: 315 - DNA, 51 bp, Artificial Sequence
  Description of Artificial Sequence: Synthetic oligonucleotide
gatcaacgtgtcaccgcctttttttttttttttttttgaagctccaaattc

SEQ ID NO: 316 - DNA, 45 bp, Artificial Sequence; identical to SEQ ID NO: 302
  Description of Artificial Sequence: Synthetic oligonucleotide

SEQ ID NO: 317 - DNA, 45 bp, Artificial Sequence; identical to SEQ ID NO: 302
  Description of Artificial Sequence: Synthetic oligonucleotide

SEQ ID NO: 318 - DNA, 45 bp, Artificial Sequence; identical to SEQ ID NO: 302
  Description of Artificial Sequence: Synthetic oligonucleotide

SEQ ID NO: 319 - DNA, 45 bp, Artificial Sequence; identical to SEQ ID NO: 302
  Description of Artificial Sequence: Synthetic oligonucleotide

SEQ ID NO: 320 - DNA, 45 bp, Artificial Sequence; identical to SEQ ID NO: 302
  Description of Artificial Sequence: Synthetic oligonucleotide

SEQ ID NO: 321 - DNA, 45 bp, Artificial Sequence; identical to SEQ ID NO: 302
  Description of Artificial Sequence: Synthetic oligonucleotide

SEQ ID NO: 322 - DNA, 41 bp, Artificial Sequence; identical to SEQ ID NO: 132
  Description of Artificial Sequence: Synthetic oligonucleotide

SEQ ID NO: 323 - DNA, 43 bp, Artificial Sequence; identical to SEQ ID NO: 133
  Description of Artificial Sequence: Synthetic oligonucleotide

SEQ ID NO: 324 - DNA, 43 bp, Artificial Sequence; identical to SEQ ID NO: 134
  Description of Artificial Sequence: Synthetic oligonucleotide

SEQ ID NO: 325 - DNA, 44 bp, Artificial Sequence; identical to SEQ ID NO: 135
  Description of Artificial Sequence: Synthetic oligonucleotide

SEQ ID NO: 326 - DNA, 44 bp, Artificial Sequence; identical to SEQ ID NO: 136
  Description of Artificial Sequence: Synthetic oligonucleotide

SEQ ID NO: 327 - DNA, 45 bp, Artificial Sequence; identical to SEQ ID NO: 137
  Description of Artificial Sequence: Synthetic oligonucleotide

SEQ ID NO: 328 - DNA, 45 bp, Artificial Sequence; identical to SEQ ID NO: 138
  Description of Artificial Sequence: Synthetic oligonucleotide

SEQ ID NO: 329 - DNA, 46 bp, Artificial Sequence; identical to SEQ ID NO: 139
  Description of Artificial Sequence: Synthetic oligonucleotide

SEQ ID NO: 330 - DNA, 46 bp, Artificial Sequence; identical to SEQ ID NO: 140
  Description of Artificial Sequence: Synthetic oligonucleotide

SEQ ID NO: 331 - DNA, 38 bp, Artificial Sequence
  Description of Artificial Sequence: Synthetic oligonucleotide
gatcaacgtgtcaccgccttttttttttttgaagctcc

SEQ ID NO: 332 - DNA, 38 bp, Artificial Sequence
  Description of Artificial Sequence: Synthetic oligonucleotide
gatcaacgtgtcaccgccttttttttttttgtagctcc

SEQ ID NO: 333 - DNA, 38 bp, Artificial Sequence
  Description of Artificial Sequence: Synthetic oligonucleotide
gatcaacgtgtcaccgccttttttttttttgacgctcc

SEQ ID NO: 334 - DNA, 38 bp, Artificial Sequence
  Description of Artificial Sequence: Synthetic oligonucleotide
gatcaacgtgtcaccgccttttttttttttgaagcgcc

SEQ ID NO: 335 - DNA, 38 bp, Artificial Sequence
  Description of Artificial Sequence: Synthetic oligonucleotide
gatcaacgtgtcaccgccttttttttttttgacgcgcc

SEQ ID NO: 336 - DNA, 38 bp, Artificial Sequence
  Description of Artificial Sequence: Synthetic oligonucleotide
gatcaacgtgtcaccgccttttttttttttgcagcgcc

SEQ ID NO: 337 - DNA, 45 bp, Artificial Sequence
  Description of Artificial Sequence: Synthetic oligonucleotide
gatcaacgtgtcaccgcctttttttttttttttttttgacgctcc

SEQ ID NO: 338 - DNA, 45 bp, Artificial Sequence
  Description of Artificial Sequence: Synthetic oligonucleotide
gatcaacgtgtcaccgcctttttttttttttttttttgaagcgcc

SEQ ID NO: 339 - DNA, 45 bp, Artificial Sequence
  Description of Artificial Sequence: Synthetic oligonucleotide
gatcaacgtgtcaccgcctttttttttttttttttttgacgcgcc

SEQ ID NO: 340 - DNA, 45 bp, Artificial Sequence
  Description of Artificial Sequence: Synthetic oligonucleotide
gatcaacgtgtcaccgcctttttttttttttttttttgcagcgcc

SEQ ID NO: 341 - DNA, 49 bp, Artificial Sequence; identical to SEQ ID NO: 151
  Description of Artificial Sequence: Synthetic oligonucleotide

SEQ ID NO: 342 - DNA, 49 bp, Artificial Sequence; identical to SEQ ID NO: 152
  Description of Artificial Sequence: Synthetic oligonucleotide

SEQ ID NO: 343 - DNA, 49 bp, Artificial Sequence; identical to SEQ ID NO: 153
  Description of Artificial Sequence: Synthetic oligonucleotide

SEQ ID NO: 344 - DNA, 49 bp, Artificial Sequence; identical to SEQ ID NO: 154
  Description of Artificial Sequence: Synthetic oligonucleotide

SEQ ID NO: 345 - DNA, 49 bp, Artificial Sequence; identical to SEQ ID NO: 155
  Description of Artificial Sequence: Synthetic oligonucleotide

SEQ ID NO: 346 - DNA, 49 bp, Artificial Sequence; identical to SEQ ID NO: 156
  Description of Artificial Sequence: Synthetic oligonucleotide

SEQ ID NO: 347 - DNA, 49 bp, Artificial Sequence; identical to SEQ ID NO: 157
  Description of Artificial Sequence: Synthetic oligonucleotide

SEQ ID NO: 348 - DNA, 49 bp, Artificial Sequence; identical to SEQ ID NO: 158
  Description of Artificial Sequence: Synthetic oligonucleotide

SEQ ID NO: 349 - DNA, 49 bp, Artificial Sequence; identical to SEQ ID NO: 151
  Description of Artificial Sequence: Synthetic oligonucleotide

SEQ ID NO: 350 - DNA, 49 bp, Artificial Sequence; identical to SEQ ID NO: 152
  Description of Artificial Sequence: Synthetic oligonucleotide

SEQ ID NO: 351 - DNA, 39 bp, Artificial Sequence
  Description of Artificial Sequence: Synthetic oligonucleotide
gatcaacgtgtcaccgccttttttttttttgaagctcca

SEQ ID NO: 352 - DNA, 39 bp, Artificial Sequence
  Description of Artificial Sequence: Synthetic oligonucleotide
gatcaacgtgtcaccgccttttttttttttgtagctcca

SEQ ID NO: 353 - DNA, 40 bp, Artificial Sequence
  Description of Artificial Sequence: Synthetic oligonucleotide
gatcaacgtgtcaccgccttttttttttttgaagctccaa

SEQ ID NO: 354 - DNA, 40 bp, Artificial Sequence
  Description of Artificial Sequence: Synthetic oligonucleotide
gatcaacgtgtcaccgccttttttttttttgtagctccaa

SEQ ID NO: 355 - DNA, 46 bp, Artificial Sequence; identical to SEQ ID NO: 309
  Description of Artificial Sequence: Synthetic oligonucleotide

SEQ ID NO: 356 - DNA, 47 bp, Artificial Sequence; identical to SEQ ID NO: 311
  Description of Artificial Sequence: Synthetic oligonucleotide

SEQ ID NO: 357 - DNA, 48 bp, Artificial Sequence; identical to SEQ ID NO: 313
  Description of Artificial Sequence: Synthetic oligonucleotide

SEQ ID NO: 358 - DNA, 50 bp, Artificial Sequence; identical to SEQ ID NO: 168
  Description of Artificial Sequence: Synthetic oligonucleotide

SEQ ID NO: 359 - DNA, 50 bp, Artificial Sequence; identical to SEQ ID NO: 169
  Description of Artificial Sequence: Synthetic oligonucleotide

SEQ ID NO: 360 - DNA, 50 bp, Artificial Sequence; identical to SEQ ID NO: 170
  Description of Artificial Sequence: Synthetic oligonucleotide

SEQ ID NO: 361 - DNA, 50 bp, Artificial Sequence; identical to SEQ ID NO: 171
  Description of Artificial Sequence: Synthetic oligonucleotide

SEQ ID NO: 362 - DNA, 45 bp, Artificial Sequence; identical to SEQ ID NO: 172
  Description of Artificial Sequence: Synthetic oligonucleotide

SEQ ID NO: 363 - DNA, 45 bp, Artificial Sequence; identical to SEQ ID NO: 48
  Description of Artificial Sequence: Synthetic oligonucleotide

SEQ ID NO: 364 - DNA, 46 bp, Artificial Sequence; identical to SEQ ID NO: 174
  Description of Artificial Sequence: Synthetic oligonucleotide

SEQ ID NO: 365 - DNA, 46 bp, Artificial Sequence; identical to SEQ ID NO: 175
  Description of Artificial Sequence: Synthetic oligonucleotide

SEQ ID NO: 366 - DNA, 44 bp, Artificial Sequence; identical to SEQ ID NO: 135
  Description of Artificial Sequence: Synthetic oligonucleotide

SEQ ID NO: 367 - DNA, 44 bp, Artificial Sequence; identical to SEQ ID NO: 136
  Description of Artificial Sequence: Synthetic oligonucleotide

SEQ ID NO: 368 - DNA, 45 bp, Artificial Sequence; identical to SEQ ID NO: 137
  Description of Artificial Sequence: Synthetic oligonucleotide

SEQ ID NO: 369 - DNA, 45 bp, Artificial Sequence; identical to SEQ ID NO: 138
  Description of Artificial Sequence: Synthetic oligonucleotide

SEQ ID NO: 370 - DNA, 47 bp, Artificial Sequence; identical to SEQ ID NO: 180
  Description of Artificial Sequence: Synthetic oligonucleotide

SEQ ID NO: 371 - DNA, 47 bp, Artificial Sequence; identical to SEQ ID NO: 181
  Description of Artificial Sequence: Synthetic oligonucleotide

SEQ ID NO: 372 - DNA, 46 bp, Artificial Sequence; identical to SEQ ID NO: 139
  Description of Artificial Sequence: Synthetic oligonucleotide

SEQ ID NO: 373 - DNA, 46 bp, Artificial Sequence; identical to SEQ ID NO: 140
  Description of Artificial Sequence: Synthetic oligonucleotide

SEQ ID NO: 374 - DNA, 47 bp, Artificial Sequence; identical to SEQ ID NO: 96
  Description of Artificial Sequence: Synthetic oligonucleotide

SEQ ID NO: 375 - DNA, 37 bp, Artificial Sequence
  Description of Artificial Sequence: Synthetic oligonucleotide
gatcaacgtgtcaccgccttttttttttttgaagctc

SEQ ID NO: 376 - DNA, 37 bp, Artificial Sequence
  Description of Artificial Sequence: Synthetic oligonucleotide
gatcaacgtgtcaccgccttttttttttttgtagctc

SEQ ID NO: 377 - DNA, 44 bp, Artificial Sequence; identical to SEQ ID NO: 187
  Description of Artificial Sequence: Synthetic oligonucleotide

SEQ ID NO: 378 - DNA, 44 bp, Artificial Sequence; identical to SEQ ID NO: 188
  Description of Artificial Sequence: Synthetic oligonucleotide

SEQ ID NO: 379 - DNA, 43 bp, Artificial Sequence; identical to SEQ ID NO: 133
  Description of Artificial Sequence: Synthetic oligonucleotide

SEQ ID NO: 380 - DNA, 43 bp, Artificial Sequence; identical to SEQ ID NO: 134
  Description of Artificial Sequence: Synthetic oligonucleotide

SEQ ID NO: 381 - DNA, 10 bp, Artificial Sequence
  Description of Artificial Sequence: Synthetic probe
  Description of Combined DNA/RNA Molecule: Synthetic probe
tguacuagga

SEQ ID NO: 382 - DNA, 18 bp, Artificial Sequence
  Description of Artificial Sequence: Synthetic probe
ggctgtaggcataaattg

SEQ ID NO: 383 - DNA, 7 bp, Artificial Sequence
  Description of Artificial Sequence: Synthetic probe
accgacc

SEQ ID NO: 384 - DNA, 34 bp, Artificial Sequence
  Description of Artificial Sequence: Synthetic probe
ttgaggcatacttcaaagactgtgtgtttaaaga

SEQ ID NO: 385 - DNA, 7 bp, Artificial Sequence
  Description of Artificial Sequence: Synthetic probe
acctgga

SEQ ID NO: 386 - DNA, 34 bp, Artificial Sequence
  Description of Artificial Sequence: Synthetic probe
tcgaagaatacatcaaagactgtgtatttaagga

SEQ ID NO: 387 - DNA, 25 bp, Artificial Sequence
  Description of Artificial Sequence: Synthetic primer
catgcaactttttcacctctgccta

SEQ ID NO: 388 - DNA, 33 bp, Artificial Sequence
  Description of Artificial Sequence: Synthetic probe
  Description of Combined DNA/RNA Molecule: Synthetic probe
  misc_feature (16)..(17): BHQ-2
ccaagctgtgccttgggtggcuuuggggcaugg

SEQ ID NO: 389 - DNA, 25 bp, Artificial Sequence
  Description of Artificial Sequence: Synthetic oligonucleotide
catgcaactttttcacctctgccta

SEQ ID NO: 390 - DNA, 33 bp, Artificial Sequence
  Description of Artificial Sequence: Synthetic oligonucleotide
ccaagctgtgccttgggtggctttggggcatgg

SEQ ID NO: 391 - DNA, 16 bp, Artificial Sequence
  Description of Artificial Sequence: Synthetic probe
ccaagctgtgccttgg

SEQ ID NO: 392 - DNA, 17 bp, Artificial Sequence
  Description of Artificial Sequence: Synthetic probe
  Description of Combined DNA/RNA Molecule: Synthetic probe
gtggcuuuggggcaugg

SEQ ID NO: 393 - DNA, 49 bp, Artificial Sequence
  Description of Artificial Sequence: Synthetic oligonucleotide
gatcaacgtgtcaccgcctattctatttttttttttttttttgatgctc

SEQ ID NO: 394 - DNA, 49 bp, Artificial Sequence
  Description of Artificial Sequence: Synthetic oligonucleotide
gatcaacgtgtcaccgcctattctatttttttttttttttttttagctc

SEQ ID NO: 395 - DNA, 49 bp, Artificial Sequence
  Description of Artificial Sequence: Synthetic oligonucleotide
gatcaacgtgtcaccgcctattctatttttttttttttttttgaagcgc

SEQ ID NO: 396 - DNA, 49 bp, Artificial Sequence
  Description of Artificial Sequence: Synthetic oligonucleotide
gatcaacgtgtcaccgcctattctatttttttttttttttttgaggctc

SEQ ID NO: 397 - DNA, 49 bp, Artificial Sequence; identical to SEQ ID NO: 393
  Description of Artificial Sequence: Synthetic oligonucleotide

SEQ ID NO: 398 - DNA, 49 bp, Artificial Sequence; identical to SEQ ID NO: 394
  Description of Artificial Sequence: Synthetic oligonucleotide

SEQ ID NO: 399 - DNA, 49 bp, Artificial Sequence; identical to SEQ ID NO: 395
  Description of Artificial Sequence: Synthetic oligonucleotide

SEQ ID NO: 400 - DNA, 49 bp, Artificial Sequence; identical to SEQ ID NO: 396
  Description of Artificial Sequence: Synthetic oligonucleotide